European Patent Application EP 4 375 654 A1, published May 29, 2024. Title: 生体分子を検出する方法及び装置. Applicant: PROVIGATE Inc. The sequence listing filed with the application follows.

SEQUENCE LISTING (5 sequences)

SEQ ID NO: 1 - DNA, 23 bp, synthetic construct
  misc_feature 1..23: note = Aptamer
  source 1..23: mol_type = other DNA
tgcggttgtagtactcgtggccg

SEQ ID NO: 2 - DNA, 51 bp, synthetic construct
  misc_feature 1..51: note = Aptamer
  source 1..51: mol_type = other DNA
aaaaaaaaaaatctaactgctgcgccgccgggaaaatactgtacggttaga

SEQ ID NO: 3 - DNA, 57 bp, synthetic construct
  misc_feature 1..57: note = Aptamer
  source 1..57: mol_type = other DNA
gcaatggtacggtacttccggatgcggaaactggctaattggtgaggctggggcggt

SEQ ID NO: 4 - DNA, 51 bp, synthetic construct
  misc_feature 1..51: note = Aptamer
  source 1..51: mol_type = other DNA
cagcaccgaccttgtgctttgggagtgctggtccaagggcgttaatggaca

SEQ ID NO: 5 - DNA, 67 bp, synthetic construct
  misc_feature 1..67: note = Aptamer
  source 1..67: mol_type = other DNA
atccagagtgacgcagcatttcatcgggtccaaaaggggctgctcgggattgcggatatggacacgt